European Patent Application EP 4 201 947 A1, published June 28, 2023. Title: Process for the backbone deprotection of oligonucleotides containing a terminal alkyl phosphonate group. Applicant: F.Hoffmann-LA Roche AG. The sequence listing filed with the application follows.

SEQUENCE LISTING (1 sequence)

SEQ ID NO: 1 - DNA, 22 bp, Oligonucleotide
uuauugugaggauuuuugucgg